European Patent Specification EP 4 048 812 B1, published December 6, 2023. Title: METHODS FOR 3' OVERHANG REPAIR. Applicant: GUARDANT HEALTH, INC. The sequence listing filed with the application follows.

SEQUENCE LISTING (3 sequences)

SEQ ID NO: 1 - DNA, 58 bp, Artificial Sequence
  TruSq Universal Adapter
aatgatacggcgaccaccgagatctacactctttccctacacgacgctcttccgatct

SEQ ID NO: 2 - DNA, 63 bp, Artificial Sequence
  TruSeq Index Adapter
  misc_feature (34)..(39): n is a, c, g, t, or u
gatcggaagagcacacgtctgaactccagtcacnnnnnnatctcgtatgccgtcttctgcttg

SEQ ID NO: 3 - DNA, 58 bp, Artificial Sequence
  Exemplary Y-shaped adapter
aatgatacggcgaccaccgagatctacactctttccctacacgacgctcttccgatcc